European Patent Application EP 4 527 400 A2, published March 26, 2025. Title: METHODS AND COMPOSITIONS FOR REDUCING CLOSTRIDIUM DIFFICILE INFECTION. Applicant: MEMORIAL SLOAN-KETTERING CANCER CENTER. Application US 089331.0158, filed October 12, 2022. The sequence listing filed with the application follows.

SEQUENCE LISTING (2 sequences)

SEQ ID NO: 1 - protein, 266 aa, Clostridium scindens
  REGION 1..266: note = 7alpha-hydroxysteroid dehydrogenase
MRLKDKVILVTASTRGIGLAIAQACAKEGAKVYMGARNLERAKARADEMNAAGGNVKYVYNDATKEETYVTMIEEIIEQEGRIDVLVNNFGSSNPKKDLGIANTDPEVFIKTVNINLKSVFIASQTAVKYMAENGGGSIINISSVGGLIPDISQIAYGTSKAAINYLTKLIAVHEARHNIRCNAVLPGMTATDAVQDNLTDDFRNFFLKHTPIQRMGLPEEIAAAVVYFASDDAAYTTGQILTVSGGFGLATPIFGDLSERSDARG

SEQ ID NO: 2 - DNA, 1305 bp, Clostridium scindens
  misc_feature 1..1305: note = 7alpha-hydroxysteroid dehydrogenase
  source 1..1305: mol_type = genomic DNA
ggccggaatgcagaagttgtccctggcgtttttatgaaggcgaccggcatgagatattgaacgagacagaccgggaacaggtatatgaagacctgttccaatggattgaagatcagaaaatgacgcagcaaaattaggacgctatacttaagaaaagtatccggataatgattacatgaatatgaaagatatctggaatactaaaaataaatcatatggagggattacacatgaggttaaaagacaaagtgattctggttacagcatccaccagaggcattggcctggctatcgctcaggcatgtgcgaaagaaggagccaaagtctacatgggcgccaggaatctggaacgcgccaaggcacgggctgacgagatgaatgcggcaggcggcaatgtaaagtatgtttacaatgatgcgacaaaagaagagacatacgtgacgatgattgaggaaatcatcgagcaagaagggcgcatagacgtgcttgtaaataatttcggctcatcaaatcccaagaaagatcttggaattgccaatacagacccggaggtattcatcaagacggtaaatatcaacctaaagagcgtatttatcgcaagccagacggctgttaagtatatggcggaaaatggaggtggaagcatcatcaatatctcatccgtaggaggcctgataccagatatctctcagattgcctatggaaccagcaaagcggcaatcaactatctgacgaaactgatagccgtacacgaggcaaggcataacatcagatgcaatgcggtacttccaggaatgacggcaacagatgcggtgcaggataatctgacggatgacttccgaaacttcttcttgaagcatacgccaattcagcgtatggggctcccggaagagatcgcggcagccgtagtatacttcgcaagcgatgatgccgcatataccacaggacagattcttaccgtatctggcggtttcggactggcaacgccgatatttggagatctgtctgaacgctcagatgcccgcgggtagaatttcatgggttaacttaatcaaaagcagaatcaggaaaagagacagccgggagcggctgtctcttttatctatagtgcgcctagcggcgcacgtttctaactttataggaaagttctcctttcggagaacttggggactaaaatagcccgctcaaaagcgggcatagtgaatcagacggtttggattaaaagatgtaaaagccctcttcaccaaaatcgtcatcatcaaggttatcaaattcatgtaagaaataatccatatccagaagttc